European Patent Application EP 4 556 005 A1, published May 21, 2025. Title: COMPOUNDS FOR TREATING FLAVIVIRUS INFECTIONS. Applicant: Leibniz-Institut für Virologie. Application EP. The sequence listing filed with the application follows.

SEQUENCE LISTING (3 sequences)

SEQ ID NO: 1 - DNA, 1215 bp, Homo sapiens
  source 1..1215: mol_type = genomic DNA
atggcggagtctgtggagcgcctgcagcagcgggtccaggagctggagcgggaacttgcccaggagaggagtctgcaggtcccgaggagcggcgacggagggggcggccgggtccgcatcgagaagatgagctcagaggtggtggattcgaatccctacagccgcttgatggcattgaaacgaatgggaattgtaagcgactatgagaaaatccgtacctttgccgtagcaatagtaggtgttggtggagtaggtagtgtgactgctgaaatgctgacaagatgtggcattggtaagttgctactctttgattatgacaaggtggaactagccaatatgaatagacttttcttccaacctcatcaagcaggattaagtaaagttcaagcagcagaacatactctgaggaacattaatcctgatgttctttttgaagtacacaactataatataaccacagtggaaaactttcaacatttcatggatagaataagtaatggtgggttagaagaaggaaaacctgttgatctagttcttagctgtgtggacaattttgaagctcgaatgacaataaatacagcttgtaatgaacttggacaaacatggatggaatctggggtcagtgaaaatgcagtttcagggcatatacagcttataattcctggagaatctgcttgttttgcgtgtgctccaccacttgtagttgctgcaaatattgatgaaaagactctgaaacgagaaggtgtttgtgcagccagtcttcctaccactatgggtgtggttgctgggatcttagtacaaaacgtgttaaagtttctgttaaattttggtactgttagtttttaccttggatacaatgcaatgcaggatttttttcctactatgtccatgaagccaaatcctcagtgtgatgacagaaattgcaggaagcagcaggaggaatataagaaaaaggtagcagcactgcctaaacaagaggttatacaagaagaggaagagataatccatgaagataatgaatggggtattgagctggtatctgaggtttcagaagaggaactgaaaaatttttcaggtccagttccagacttacctgaaggaattacagtggcatacacaattccaaaaaagcaagaagattctgtcactgagttaacagtggaagattctggtgaaagcttggaagacctcatggccaaaatgaagaatatgtag

SEQ ID NO: 2 - protein, 404 aa, Homo sapiens
MAESVERLQQRVQELERELAQERSLQVPRSGDGGGGRVRIEKMSSEVVDSNPYSRLMALKRMGIVSDYEKIRTFAVAIVGVGGVGSVTAEMLTRCGIGKLLLFDYDKVELANMNRLFFQPHQAGLSKVQAAEHTLRNINPDVLFEVHNYNITTVENFQHFMDRISNGGLEEGKPVDLVLSCVDNFEARMTINTACNELGQTWMESGVSENAVSGHIQLIIPGESACFACAPPLVVAANIDEKTLKREGVCAASLPTTMGVVAGILVQNVLKFLLNFGTVSFYLGYNAMQDFFPTMSMKPNPQCDDRNCRKQQEEYKKKVAALPKQEVIQEEEEIIHEDNEWGIELVSEVSEEELKNFSGPVPDLPEGITVAYTIPKKQEDSVTELTVEDSGESLEDLMAKMKNM

SEQ ID NO: 3 - protein, 348 aa, Homo sapiens
MALKRMGIVSDYEKIRTFAVAIVGVGGVGSVTAEMLTRCGIGKLLLFDYDKVELANMNRLFFQPHQAGLSKVQAAEHTLRNINPDVLFEVHNYNITTVENFQHFMDRISNGGLEEGKPVDLVLSCVDNFEARMTINTACNELGQTWMESGVSENAVSGHIQLIIPGESACFACAPPLVVAANIDEKTLKREGVCAASLPTTMGVVAGILVQNVLKFLLNFGTVSFYLGYNAMQDFFPTMSMKPNPQCDDRNCRKQQEEYKKKVAALPKQEVIQEEEEIIHEDNEWGIELVSEVSEEELKNFSGPVPDLPEGITVAYTIPKKQEDSVTELTVEDSGESLEDLMAKMKNM